European Patent Application EP 4 726 045 A1, published April 15, 2026. Title: 表达盒组合及其应用. Applicant: 北京中因科技有限公司. Application CN. The sequence listing filed with the application follows.

SEQUENCE LISTING (70 sequences)

SEQ ID NO: 1 - protein, 2273 aa, Homo sapiens [sequence omitted]

SEQ ID NO: 2 - DNA, 6822 bp, Homo sapiens
  source 1..6822: mol_type = genomic DNA
atgggcttcgtgagacagatacagcttttgctctggaagaactggaccctgcggaaaaggcaaaagattcgctttgtggtggaactcgtgtggcctttatctttatttctggtcttgatctggttaaggaatgccaacccactctacagccatcatgaatgccatttccccaacaaggcgatgccctcagcaggaatgctgccgtggctccaggggatcttctgcaatgtgaacaatccctgttttcaaagccccaccccaggagaatctcctggaattgtgtcaaactataacaactccatcttggcaagggtatatcgagattttcaagaactcctcatgaatgcaccagagagccagcaccttggccgtatttggacagagctacacatcttgtcccaattcatggacaccctccggactcacccggagagaattgcaggaagaggaatacgaataagggatatcttgaaagatgaagaaacactgacactatttctcattaaaaacatcggcctgtctgactcagtggtctaccttctgatcaactctcaagtccgtccagagcagttcgctcatggagtcccggacctggcgctgaaggacatcgcctgcagcgaggccctcctggagcgcttcatcatcttcagccagagacgcggggcaaagacggtgcgctatgccctgtgctccctctcccagggcaccctacagtggatagaagacactctgtatgccaacgtggacttcttcaagctcttccgtgtgcttcccacactcctagacagccgttctcaaggtatcaatctgagatcttggggaggaatattatctgatatgtcaccaagaattcaagagtttatccatcggccgagtatgcaggacttgctgtgggtgaccaggcccctcatgcagaatggtggtccagagacctttacaaagctgatgggcatcctgtctgacctcctgtgtggctaccccgagggaggtggctctcgggtgctctccttcaactggtatgaagacaataactataaggcctttctggggattgactccacaaggaaggatcctatctattcttatgacagaagaacaacatccttttgtaatgcattgatccagagcctggagtcaaatcctttaaccaaaatcgcttggagggcggcaaagcctttgctgatgggaaaaatcctgtacactcctgattcacctgcagcacgaaggatactgaagaatgccaactcaacttttgaagaactggaacacgttaggaagttggtcaaagcctgggaagaagtagggccccagatctggtacttctttgacaacagcacacagatgaacatgatcagagataccctggggaacccaacagtaaaagactttttgaataggcagcttggtgaagaaggtattactgctgaagccatcctaaacttcctctacaagggccctcgggaaagccaggctgacgacatggccaacttcgactggagggacatatttaacatcactgatcgcaccctccgcctggtcaatcaatacctggagtgcttggtcctggataagtttgaaagctacaatgatgaaactcagctcacccaacgtgccctctctctactggaggaaaacatgttctgggccggagtggtattccctgacatgtatccctggaccagctctctaccaccccacgtgaagtataagatccgaatggacatagacgtggtggagaaaaccaataagattaaagacaggtattgggattctggtcccagagctgatcccgtggaagatttccggtacatctggggcgggtttgcctatctgcaggacatggttgaacaggggatcacaaggagccaggtgcaggcggaggctccagttggaatctacctccagcagatgccctacccctgcttcgtggacgattctttcatgatcatcctgaaccgctgtttccctatcttcatggtgctggcatggatctactctgtctccatgactgtgaagagcatcgtcttggagaaggagttgcgactgaaggagaccttgaaaaatcagggtgtctccaatgcagtgatttggtgtacctggttcctggacagcttctccatcatgtcgatgagcatcttcctcctgacgatattcatcatgcatggaagaatcctacattacagcgacccattcatcctcttcctgttcttgttggctttctccactgccaccatcatgctgtgctttctgctcagcaccttcttctccaaggccagtctggcagcagcctgtagtggtgtcatctatttcaccctctacctgccacacatcctgtgcttcgcctggcaggaccgcatgaccgctgagctgaagaaggctgtgagcttactgtctccggtggcatttggatttggcactgagtacctggttcgctttgaagagcaaggcctggggctgcagtggagcaacatcgggaacagtcccacggaaggggacgaattcagcttcctgctgtccatgcagatgatgctccttgatgctgctgtctatggcttactcgcttggtaccttgatcaggtgtttccaggagactatggaaccccacttccttggtactttcttctacaagagtcgtattggcttggcggtgaagggtgttcaaccagagaagaaagagccctggaaaagaccgagcccctaacagaggaaacggaggatccagagcacccagaaggaatacacgactccttctttgaacgtgagcatccagggtgggttcctggggtatgcgtgaagaatctggtaaagatttttgagccctgtggccggccagctgtggaccgtctgaacatcaccttctacgagaaccagatcaccgcattcctgggccacaatggagctgggaaaaccaccaccttgtccatcctgacgggtctgttgccaccaacctctgggactgtgctcgttgggggaagggacattgaaaccagcctggatgcagtccggcagagccttggcatgtgtccacagcacaacatcctgttccaccacctcacggtggctgagcacatgctgttctatgcccagctgaaaggaaagtcccaggaggaggcccagctggagatggaagccatgttggaggacacaggcctccaccacaagcggaatgaagaggctcaggacctatcaggtggcatgcagagaaagctgtcggttgccattgcctttgtgggagatgccaaggtggtgattctggacgaacccacctctggggtggacccttactcgagacgctcaatctgggatctgctcctgaagtatcgctcaggcagaaccatcatcatgtccactcaccacatggacgaggccgacctccttggggaccgcattgccatcattgcccagggaaggctctactgctcaggcaccccactcttcctgaagaactgctttggcacaggcttgtacttaaccttggtgcgcaagatgaaaaacatccagagccaaaggaaaggcagtgaggggacctgcagctgctcgtctaagggtttctccaccacgtgtccagcccacgtcgatgacctaactccagaacaagtcctggatggggatgtaaatgagctgatggatgtagttctccaccatgttccagaggcaaagctggtggagtgcattggtcaagaacttatcttccttcttccaaataagaacttcaagcacagagcatatgccagccttttcagagagctggaggagacgctggctgaccttggtctcagcagttttggaatttctgacactcccctggaagagatttttctgaaggtcacggaggattctgattcaggacctctgtttgcgggtggcgctcagcagaaaagagaaaacgtcaacccccgacacccctgcttgggtcccagagagaaggctggacagacaccccaggactccaatgtctgctccccaggggcgccggctgctcacccagagggccagcctcccccagagccagagtgcccaggcccgcagctcaacacggggacacagctggtcctccagcatgtgcaggcgctgctggtcaagagattccaacacaccatccgcagccacaaggacttcctggcgcagatcgtgctcccggctacctttgtgtttttggctctgatgctttctattgttatccctccttttggcgaataccccgctttgacccttcacccctggatatatgggcagcagtacaccttcttcagcatggatgaaccaggcagtgagcagttcacggtacttgcagacgtcctcctgaataagccaggctttggcaaccgctgcctgaaggaagggtggcttccggagtacccctgtggcaactcaacaccctggaagactccttctgtgtccccaaacatcacccagctgttccagaagcagaaatggacacaggtcaacccttcaccatcctgcaggtgcagcaccagggagaagctcaccatgctgccagagtgccccgagggtgccgggggcctcccgcccccccagagaacacagcgcagcacggaaattctacaagacctgacggacaggaacatctccgacttcttggtaaaaacgtatcctgctcttataagaagcagcttaaagagcaaattctgggtcaatgaacagaggtatggaggaatttccattggaggaaagctcccagtcgtccccatcacgggggaagcacttgttgggtttttaagcgaccttggccggatcatgaatgtgagcgggggccctatcactagagaggcctctaaagaaatacctgatttccttaaacatctagaaactgaagacaacattaaggtgtggtttaataacaaaggctggcatgccctggtcagctttctcaatgtggcccacaacgccatcttacgggccagcctgcctaaggacaggagccccgaggagtatggaatcaccgtcattagccaacccctgaacctgaccaaggagcagctctcagagattacagtgctgaccacttcagtggatgctgtggttgccatctgcgtgattttctccatgtccttcgtcccagccagctttgtcctttatttgatccaggagcgggtgaacaaatccaagcacctccagtttatcagtggagtgagccccaccacctactgggtgaccaacttcctctgggacatcatgaattattccgtgagtgctgggctggtggtgggcatcttcatcgggtttcagaagaaagcctacacttctccagaaaaccttcctgcccttgtggcactgctcctgctgtatggatgggcggtcattcccatgatgtacccagcatccttcctgtttgatgtccccagcacagcctatgtggctttatcttgtgctaatctgttcatcggcatcaacagcagtgctattaccttcatcttggaattatttgagaataaccggacgctgctcaggttcaacgccgtgctgaggaagctgctcattgtcttcccccacttctgcctgggccggggcctcattgaccttgcactgagccaggctgtgacagatgtctatgcccggtttggtgaggagcactctgcaaatccgttccactgggacctgattgggaagaacctgtttgccatggtggtggaaggggtggtgtacttcctcctgaccctgctggtccagcgccacttcttcctctcccaatggattgccgagcccactaaggagcccattgttgatgaagatgatgatgtggctgaagaaagacaaagaattattactggtggaaataaaactgacatcttaaggctacatgaactaaccaagatttatccaggcacctccagcccagcagtggacaggctgtgtgtcggagttcgccctggagagtgctttggcctcctgggagtgaatggtgccggcaaaacaaccacattcaagatgctcactggggacaccacagtgacctcaggggatgccaccgtagcaggcaagagtattttaaccaatatttctgaagtccatcaaaatatgggctactgtcctcagtttgatgcaattgatgagctgctcacaggacgagaacatctttacctttatgcccggcttcgaggtgtaccagcagaagaaatcgaaaaggttgcaaactggagtattaagagcctgggcctgactgtctacgccgactgcctggctggcacgtacagtgggggcaacaagcggaaactctccacagccatcgcactcattggctgcccaccgctggtgctgctggatgagcccaccacagggatggacccccaggcacgccgcatgctgtggaacgtcatcgtgagcatcatcagagaagggagggctgtggtcctcacatcccacagcatggaagaatgtgaggcactgtgtacccggctggccatcatggtaaagggcgcctttcgatgtatgggcaccattcagcatctcaagtccaaatttggagatggctatatcgtcacaatgaagatcaaatccccgaaggacgacctgcttcctgacctgaaccctgtggagcagttcttccaggggaacttcccaggcagtgtgcagagggagaggcactacaacatgctccagttccaggtctcctcctcctccctggcgaggatcttccagctcctcctctcccacaaggacagcctgctcatcgaggagtactcagtcacacagaccacactggaccaggtgtttgtaaattttgctaaacagcagactgaaagtcatgacctccctctgcaccctcgagctgctggagccagtcgacaagcccaggactga

SEQ ID NO: 3 - DNA, 6822 bp, synthetic construct
  source 1..6822: mol_type = other DNA
atgggattcgtgcggcagatccagcttctgctctggaagaattggaccctgcgtaaacggcagaagattagatttgtggtggagctggtgtggcctctgagcctgttcttggtgctgatctggctgcgaaacgccaaccctctgtactcccaccatgagtgtcacttccctaacaaggccatgccttctgctggcatgctgccttggctgcagggcatcttctgcaacgtgaacaacccctgcttccagagccccacccctggagagtctcccggcatcgtcagtaactacaacaactccatcctcgccagagtgtacagagatttccaggagctgctgatgaacgcccctgagtctcaacacctggggagaatctggaccgagctccatatactgtcacagttcatggataccctacggacccaccccgaacggatcgccggcagaggcattagaatccgggatatccttaaggacgaagagacactgactctttttctgattaagaatatcggattgtctgattcggtggtgtacctgctgatcaacagccaggtgagacctgagcagttcgcccacggcgtgcctgacttagcgctgaaggacattgcctgctctgaggccttgctggaaagattcatcatcttctctcagcggcggggggccaagacagttcggtacgccctgtgcagcctgagccagggcaccttgcagtggatcgaagacaccctgtatgctaacgtggacttctttaaactgtttagagtgttgccaaccttactggacagccggagccagggcatcaacctgagatcctggggtggaatcctgagcgatatgagccccagaatccaggagttcatccaccggcctagcatgcaggacttgctgtgggtgactcgtcccctgatgcaaaacggaggaccagaaacatttacaaagcttatgggcatcctgagcgacctcttgtgcggctaccctgagggcggcggcagccgggtgttaagctttaactggtacgaggacaacaactacaaggccttccttggtatcgatagcacacgaaaggacccaatctacagctacgaccgtagaacaaccagtttctgcaacgccctgatccagtcccttgaatctaatcctttgacaaagatcgcttggcgggccgccaagcctctgctgatgggcaagatcctgtacacccctgacagccctgccgccagaagaatcctaaagaatgccaacagcactttcgaggaactcgaacacgtgcggaagctggtcaaagcctgggaggaggtgggccctcaaatctggtacttcttcgataactccacccagatgaacatgatcagagacaccttgggaaatccgaccgtgaaggacttcctgaatagacagctaggtgaggagggaatcaccgccgaggccatcctgaactttctgtacaaaggccctcgggagtcccaggctgatgacatggccaattttgactggagagacatattcaacatcacagaccgtacccttagactggtgaaccagtacctggaatgcttagtcctggataagttcgaaagctacaacgacgagacccagctgacccaacgggcactgtctctactggaggagaatatgttctgggccggtgtggtgttccctgacatgtacccctggacaagcagcctgccacctcacgtgaaatacaagatccggatggacattgacgtggtggaaaagacaaacaagatcaaggacagatactgggacagcggacctagggccgatcctgtggaggatttccggtacatctggggtggcttcgcttacctgcaggacatggtggaacagggcatcacgagaagccaggtgcaggctgaggcccctgtgggaatctacctccaacagatgccctacccctgcttcgtggacgacagcttcatgatcatcctgaatagatgtttcccaatcttcatggtgctggcctggatctacagcgtgtccatgactgtgaagtccatcgtgctggagaaggagctgcggctaaaagagactctgaagaatcagggcgtgagcaacgccgtaatctggtgcacctggttcctggactccttctccatcatgagcatgagcatcttcctactgacaatctttatcatgcacggcagaattctgcactacagcgaccctttcatcctgtttctttttttgctggctttcagcaccgccaccatcatgctgtgcttcctgttaagcaccttcttctcaaaggccagcctagctgcagcatgctccggcgtcatctactttactttatacctgccccacatcctgtgtttcgcctggcaggacagaatgacagccgagctgaaaaaggccgtatccctgttgagccccgtggccttcgggtttggaaccgagtacctggtacggttcgaggaacaaggcctgggcctgcagtggtccaacatcggcaactcgccgaccgagggcgacgaattcagcttcctgctgtccatgcagatgatgctgctggatgccgcagtgtatggcctcctggcttggtacttggaccaggtgttccccggcgactacgggactccactgccatggtactttctgctgcaggagagctactggctgggcggcgagggctgcagcaccagagaggaaagagccctggagaagacagagcctctgactgaagaaaccgaagaccctgagcaccctgaggggatacacgactcttttttcgagagggaacatcctggatgggtccctggcgtttgcgtgaagaacctggtgaagatcttcgagccttgtggcaggccagccgtggatagactgaatatcaccttctacgagaaccagatcaccgccttcctgggccacaacggcgcgggaaagaccacaactctgagcatcctgaccggactgctgcctccaacttccggcaccgtgctcgtcggcggcagggacatcgagaccagtctggacgccgtgagacagagcctcggcatgtgccctcagcacaatatcctgtttcaccacttaaccgttgcagaacacatgctgttctacgcccagttaaaaggcaagtcgcaggaggaggcccagctggagatggaagcaatgctcgaagatacaggcctgcaccataagagaaacgaagaggcccaggatctctccggcggcatgcagagaaaactgagcgtagccatcgccttcgtgggagatgcaaaggtggtaatcctagatgagcctacatctggggtggacccgtacagccggcgcagtatttgggatttactgctgaagtacagaagcggtagaaccatcatcatgtctacccaccacatggacgaggctgatctgctgggagatcggatcgccataatcgcccagggaagactgtattgcagcggcacaccactgttcctcaaaaactgctttgggacgggactgtacctgacgctggtccggaaaatgaagaacatccagtcccagagaaagggctctgaagggacctgttcttgcagctctaagggcttcagtaccacctgccctgcccacgtggacgacctgactcccgaacaggtgctggacggcgatgtgaacgagctgatggacgtggtgctgcatcacgtacccgaagccaagctggttgaatgcatcggccaggagctcattttccttcttcctaacaagaacttcaagcacagagcttatgcctctctgttcagggaactggaggaaaccctagccgacctgggtctgtctagcttcggcatctctgacacacctctggaggagatctttctgaaagtgactgaggattctgatagcggaccactgttcgccggaggcgctcagcagaagagagaaaacgtcaatcctagacacccttgtctgggaccgagagagaaggccggccagacccctcaagattccaatgtgtgtagccctggcgcccccgctgctcacccagagggccagcctcctcctgaacctgaatgccccggcccccagctgaacaccggcactcagctggtcctgcagcacgtgcaggccctgctggtgaagcgcttccagcacacaatccgcagtcataaagacttcctcgctcagatcgtgctcccggctacattcgtgtttctggccctcatgctgtctatcgtgatcccacctttcggcgaataccctgcgctgaccctgcacccctggatatacggtcagcaatacacctttttcagcatggacgagcccggaagcgagcagttcaccgtgctggccgatgtgctgctgaacaagcctggcttcggcaaccggtgcctgaaagaaggatggctgccagagtacccctgcggcaatagcacaccttggaagacccctagcgtgtcccctaacatcacccagctgtttcaaaaacagaaatggacccaagtgaatccttcaccttcatgcagatgttctacacgtgaaaagctgaccatgttacccgagtgtcctgaaggagctggcggccttcctcctccccagaggacccagagaagcaccgaaatcctgcaggacctgacagaccggaacatctccgactttcttgtcaagacctaccctgccctgattaggagtagcctgaaatctaagttttgggttaatgaacagcggtacggcggcatcagcatcggcggtaagctgcccgtggtgcctattacaggcgaggccctggtgggcttcctcagtgatttgggacggataatgaacgtgagtggcggcccaatcacacgggaagccagcaaagagatccctgatttcctgaagcacctggaaacagaggataatataaaggtgtggttcaacaacaaaggctggcacgccctggtgagtttcctcaacgtagcccacaacgctatcctgagagcctctctacctaaggacagaagccccgaagagtacggcattaccgtgatcagccagcccctaaacctgacaaaggaacagctgagcgagattaccgtcctgacaacctccgttgacgcggtggtggcgatctgcgtgatcttttctatgagcttcgtgcctgccagcttcgtgctgtacctgatccaggagagagtgaacaagagcaagcacctgcaatttatttctggcgtgagcccaaccacctactgggtgaccaacttcctgtgggacatcatgaactacagcgtgtctgccggcctggtggtaggcatcttcatcggcttccagaagaaggcctacacctctcctgagaatctgcctgctctcgtggccctgctgctgctgtacggctgggccgtgatccccatgatgtaccccgctagcttcttatttgacgtgccctcaacagcatacgtggccttatcctgcgccaacctgtttataggaatcaattctagcgccatcacgttcatcctagaactgttcgagaacaaccggacactgctgcgattcaacgccgtcctgcggaagctcctgattgtgttccctcatttctgtctgggcagagggctgatcgacctggccctgagccaagccgtgaccgatgtgtacgcgagattcggcgaggagcactccgccaaccctttccactgggacctgatcggcaagaatctgttcgccatggttgtggagggtgtggtgtacttcctgcttacactgctggtgcagagacacttcttcctgtcccagtggattgccgaacccaccaaggaacccatcgtcgacgaggatgacgacgtggccgaggagagacagagaatcatcaccggcgggaacaaaaccgacatcctgagactccacgagctgacaaagatctatcctggcacaagcagccccgccgtggatcggctgtgtgtgggcgtcagacctggcgagtgcttcggcctgctgggcgtgaacggcgccggcaagaccacaaccttcaagatgctgaccggcgacaccacggtgacctccggcgacgccacagtggccggcaaaagcatcctcacaaacatctccgaagtgcaccagaacatgggctactgcccccagtttgatgctatagacgagctgttgaccggtagagaacacctgtacctgtacgccagactgagaggcgtgcctgctgaagagatcgaaaaggtggcaaactggagcatcaagtcactgggcctgacagtctacgccgactgcctggccggcacgtactctggcggcaataagcggaaactgagcaccgccattgccttgattggatgtccgcctctggtgctgctggacgagccgacaacaggcatggacccccaagcccggagaatgctgtggaacgtgatcgtgagcataatcagagagggcagagccgtggttttgacttctcacagcatggaagaatgtgaagcgctctgcacccggcttgccatcatggtcaaaggcgccttccggtgcatgggcaccattcagcacctgaagtccaagttcggcgacggctacatcgtgacaatgaagatcaaatctcccaaggacgacctgcttccagatctgaaccctgtggaacagttcttccagggaaatttccctggaagcgtgcagagagagagacactacaatatgctgcagtttcaggtaagcagcagcagccttgctcggatctttcagctgctgcttagccacaaggactctctgctgatcgaagagtacagcgtgacccagacaacgcttgatcaggtgttcgtgaacttcgccaagcagcaaaccgagagccatgatctgcctcttcacccacgagctgccggcgccagcagacaggcccaggactga

SEQ ID NO: 4 - protein, 140 aa, unidentified
CLSYETEILTVEYGLLPIGKIVEKRIECTVYSVDNNGNIYTQPVAQWHDRGEQEVFEYCLEDGSLIRATKDHKFMTVDGQMLPIDEIFERELDLMRVDNLPNIKIATRKYLGKQNVYDIGVERDHNFALKNGFIASNCFN

SEQ ID NO: 5 - protein, 126 aa, unidentified
CLDLKTQVQTPQGMKEISNIQVGDLVLSNTGYNEVLNVFPKSKKKSYKITLEDGKEIICSEEHLFPTQTGEMNISGGLKEGMCLYVKEMMLKKILKIEELDERELIDIEVSGNHLFYANDILTHNS

SEQ ID NO: 6 - protein, 134 aa, unidentified
CLSLDTMVVTNGKAIEIRDVKVGDWLESECGPVQVTEVLPIIKQPVFEIVLKSGKKIRVSANHKFPTKDGLKTINSGLKVGDFLRSRAKMCEIFENEIDWDEIASIEYVGVEETIDINVTNDRLFFANGILTHN

SEQ ID NO: 7 - protein, 145 aa, unidentified
CLVGSSEIITRNYGKTTIKEVVEIFDNDKNIQVLAFNTHTDNIEWAPIKAAQLTRPNAELVELEIDTLHGVKTIRCTPDHPVYTKNRGYVRADELTDDDELVVAIMEAKTYIGKLKSRKIVSNEDTYDIQTSTHNFFANDILVHN

SEQ ID NO: 8 - protein, 141 aa, unidentified
CFVPGTLVNTENGLKKIEEIKVGDKVFSHTGKLQEVVDTLIFDRDEEIISINGIDCTKNHEFYVIDKENANRVNEDNIHLFARWVHAEELDMKKHLLIELEMKFKLKEITSIETKHYKGKVHDLTVNQDHSYNVRGTVVHN

SEQ ID NO: 9 - protein, 157 aa, unidentified
CFSGDTLVALTDGRSVSFEQLVEEEKQGKQNFCYTIRHDGSIGVEKIINARKTKTNAKVIKVTLDNGESIICTPDHKFMLRDGSYKCAMDLTLDDSLMPLHRKISTTEDSGHAMEAVLNYNHRIVNIEAVSETIDVYDIEVPHTHNFALASGVFVHN

SEQ ID NO: 10 - protein, 178 aa, unidentified
ALAYDEPIYLSDGNIINIGEFVDKFFKKYKNSIKKEDNGFGWIDIGNENIYIKSFNKLSLIIEDKRILRVWRKKYSGKLIKITTKNRREITLTHDHPVYISKTGEVLEINAEMVKVGDYIYIPKNNTGSAGSAAGSGINLDEVIKVETVDYNGHIYDLTVEDNHTYIAGKNEGFAVSN

SEQ ID NO: 11 - protein, 147 aa, unidentified
CLSYETEILTVEYGSLPIGKIVEKRIECTVYSVDNNGNIYTQPVAQWHDRGEQEVFEYCLEDGSLIRATKDHKFMTVDGQMLPIDEIFERELDLMRVDNLPNGSAGSAAGSGVKVIGRRSLGVQRIFDIGLRQDHNFLLANGAIAAN

SEQ ID NO: 12 - protein, 9 aa, unidentified
YPYDVPDYA

SEQ ID NO: 13 - protein, 8 aa, unidentified
DYKDDDDK

SEQ ID NO: 14 - protein, 104 aa, unidentified
GRKNIILSSQPSTDDRVTWVKSVDEAIAACGDVPEIMVIGGGRVIEQFLPKAQKLYLTHIDAEVEGDTHFPDYEPDDWESVFSEFHDADAQNSHSYCFEILERR

SEQ ID NO: 15 - protein, 102 aa, unidentified
CLSYETEILTVEYGLLPIGKIVEKRIECTVYSVDNNGNIYTQPVAQWHDRGEQEVFEYCLEDGSLIRATKDHKFMTVDGQMLPIDEIFERELDLMRVDNLPN

SEQ ID NO: 16 - protein, 38 aa, unidentified
IKIATRKYLGKQNVYDIGVERDHNFALKNGFIASNCFN

SEQ ID NO: 17 - protein, 88 aa, unidentified
CLDLKTQVQTPQGMKEISNIQVGDLVLSNTGYNEVLNVFPKSKKKSYKITLEDGKEIICSEEHLFPTQTGEMNISGGLKEGMCLYVKE

SEQ ID NO: 18 - protein, 38 aa, unidentified
MMLKKILKIEELDERELIDIEVSGNHLFYANDILTHNS

SEQ ID NO: 19 - protein, 89 aa, unidentified
CLSLDTMVVTNGKAIEIRDVKVGDWLESECGPVQVTEVLPIIKQPVFEIVLKSGKKIRVSANHKFPTKDGLKTINSGLKVGDFLRSRAK

SEQ ID NO: 20 - protein, 45 aa, unidentified
MCEIFENEIDWDEIASIEYVGVEETIDINVTNDRLFFANGILTHN

SEQ ID NO: 21 - protein, 105 aa, unidentified
CLVGSSEIITRNYGKTTIKEVVEIFDNDKNIQVLAFNTHTDNIEWAPIKAAQLTRPNAELVELEIDTLHGVKTIRCTPDHPVYTKNRGYVRADELTDDDELVVAI

SEQ ID NO: 22 - protein, 40 aa, unidentified
MEAKTYIGKLKSRKIVSNEDTYDIQTSTHNFFANDILVHN

SEQ ID NO: 23 - protein, 101 aa, unidentified
CFVPGTLVNTENGLKKIEEIKVGDKVFSHTGKLQEVVDTLIFDRDEEIISINGIDCTKNHEFYVIDKENANRVNEDNIHLFARWVHAEELDMKKHLLIELE

SEQ ID NO: 24 - protein, 40 aa, unidentified
MKFKLKEITSIETKHYKGKVHDLTVNQDHSYNVRGTVVHN

SEQ ID NO: 25 - protein, 113 aa, unidentified
CFSGDTLVALTDGRSVSFEQLVEEEKQGKQNFCYTIRHDGSIGVEKIINARKTKTNAKVIKVTLDNGESIICTPDHKFMLRDGSYKCAMDLTLDDSLMPLHRKISTTEDSGHA

SEQ ID NO: 26 - protein, 44 aa, unidentified
MEAVLNYNHRIVNIEAVSETIDVYDIEVPHTHNFALASGVFVHN

SEQ ID NO: 27 - protein, 12 aa, unidentified
ALAYDEPIYLSD

SEQ ID NO: 28 - protein, 166 aa, unidentified
GNIINIGEFVDKFFKKYKNSIKKEDNGFGWIDIGNENIYIKSFNKLSLIIEDKRILRVWRKKYSGKLIKITTKNRREITLTHDHPVYISKTGEVLEINAEMVKVGDYIYIPKNNTGSAGSAAGSGINLDEVIKVETVDYNGHIYDLTVEDNHTYIAGKNEGFAVSN

SEQ ID NO: 29 - protein, 133 aa, unidentified
CLSYETEILTVEYGSLPIGKIVEKRIECTVYSVDNNGNIYTQPVAQWHDRGEQEVFEYCLEDGSLIRATKDHKFMTVDGQMLPIDEIFERELDLMRVDNLPNGSAGSAAGSGVKVIGRRSLGVQRIFDIGLRQ

SEQ ID NO: 30 - protein, 14 aa, unidentified
DHNFLLANGAIAAN

SEQ ID NO: 31 - DNA, 306 bp, unidentified
  source 1..306: mol_type = other DNA
tgtctctcctacgagacagagatcctgacagtggaatatggactgctgcccattggaaaaatcgtggaaaagcggatcgagtgcaccgtctacagcgttgataacaacggcaacatctacacccaacctgtggcccagtggcacgatagaggcgaacaggaggtgttcgagtactgcctggaagatggctctctgatcagagccaccaaggaccacaagttcatgaccgtggacggccagatgctgccaatcgacgagatcttcgagagagagctggacctgatgagagtggacaatctgcctaat

SEQ ID NO: 32 - DNA, 114 bp, unidentified
  source 1..114: mol_type = other DNA
atcaagatcgctacaaggaagtacctgggcaaacagaacgtgtacgacatcggcgtggaacgggaccacaacttcgccctgaagaacggcttcatcgccagcaactgctttaac

SEQ ID NO: 33 - DNA, 264 bp, unidentified
  source 1..264: mol_type = other DNA
tgtctggatctgaagacccaggtccagacccctcagggcatgaaagagatcagcaacatccaggtgggcgacctggtgctgtctaataccggctacaacgaggtgctgaacgtgttccccaagagcaagaagaaaagctataagatcaccctggaagatggcaaggaaatcatctgcagcgaggaacacctgtttcctacacaaacaggcgagatgaacatctctggcggactgaaggaaggcatgtgcctgtacgtgaaggag

SEQ ID NO: 34 - DNA, 114 bp, unidentified
  source 1..114: mol_type = other DNA
atgatgctgaaaaagatcctgaagattgaggaactggacgagagagagctgatcgacatcgaggtgtccggaaatcacctgttctacgccaacgacatcctcacccacaacagc

SEQ ID NO: 35 - DNA, 267 bp, unidentified
  source 1..267: mol_type = other DNA
tgtctgagcctggacaccatggtggtgacaaacggcaaggccatcgagatcagagatgtgaaggttggagattggctggaatctgaatgcggccccgtgcaggtgaccgaggtgctgcctatcatcaagcagcctgtctttgagattgtgctgaaaagcggaaaaaagatccgggtgtccgctaatcacaagttcccaacaaaggacggcctcaagaccatcaacagcggcctgaaggtgggcgacttcctgagaagcagagccaag

SEQ ID NO: 36 - DNA, 135 bp, unidentified
  source 1..135: mol_type = other DNA
atgtgcgaaatcttcgagaacgagattgattgggacgaaatcgccagcatcgagtacgtgggcgtggaagagacaatcgacatcaacgtgaccaacgacagactgtttttcgccaatggcatcctgacccacaac

SEQ ID NO: 37 - DNA, 315 bp, unidentified
  source 1..315: mol_type = other DNA
tgtctggttggatctagcgagattatcacaagaaactacggcaagaccacaatcaaggaggtggtggaaatcttcgacaacgacaagaacatccaggtgctggccttcaacacccacaccgataatatcgagtgggctcctatcaaagccgctcagctgaccagaccaaacgccgagctcgtggaactggaaatcgacaccctgcacggcgtgaagacaatccggtgcacccctgaccaccccgtgtacaccaagaatagaggctacgtgcgggccgacgagctgacagacgatgatgagctggtcgtggccatc

SEQ ID NO: 38 - DNA, 120 bp, unidentified
  source 1..120: mol_type = other DNA
atggaagccaagacatacatcggcaagctgaaaagcagaaagatcgtgtctaacgaggacacctacgacatccagaccagcacccacaacttcttcgccaatgatatcctggtgcacaac

SEQ ID NO: 39 - DNA, 303 bp, unidentified
  source 1..303: mol_type = other DNA
tgttttgtgcctggaacactggtgaataccgagaacggcctgaagaaaatcgaggaaatcaaggtgggcgataaggtgttctctcatacaggcaagctgcaggaggtggtggacaccctgatcttcgaccgggacgaggaaatcatcagcatcaacggcatcgactgcaccaagaaccacgagttctacgtgatcgataaggaaaacgctaatagagtgaacgaggacaacatccacctcttcgccagatgggtccacgccgaggaactggatatgaaaaagcacctgctgattgagctggaa

SEQ ID NO: 40 - DNA, 120 bp, unidentified
  source 1..120: mol_type = other DNA
atgaaattcaagctgaaggaaatcacctctatcgagacaaagcactacaagggcaaggtgcacgatctgaccgtgaaccaggaccacagctacaacgtcagaggcaccgtggtgcataat

SEQ ID NO: 41 - DNA, 339 bp, unidentified
  source 1..339: mol_type = other DNA
tgttttagcggcgacaccctggtcgccctgacagatggaagaagcgtgtccttcgagcagctggtggaagaggaaaaacagggcaagcagaacttctgctacaccatccggcacgacggctctatcggcgtggaaaagatcattaacgctagaaagaccaagacaaacgccaaggtgatcaaggtgaccctggataatggcgagagcatcatctgcacccctgatcataagttcatgctgcgggacggaagctacaagtgcgccatggacctgacactcgacgacagcctgatgcccctgcacagaaaaatcagcaccaccgaggactctggccacgcc

SEQ ID NO: 42 - DNA, 132 bp, unidentified
  source 1..132: mol_type = other DNA
atggaagctgtgctgaactacaaccacagaatcgtgaacatcgaagccgtcagcgagacaatcgatgtgtacgacatcgaggtgcctcacacccacaacttcgccctggcctctggcgtgttcgtgcataat

SEQ ID NO: 43 - DNA, 36 bp, unidentified
  source 1..36: mol_type = other DNA
gccctggcctacgacgagcctatctacctgagcgat

SEQ ID NO: 44 - DNA, 498 bp, unidentified
  source 1..498: mol_type = other DNA
ggaaatatcatcaatattggcgagttcgtggataagttcttcaagaaatacaagaacagcatcaaaaaggaagataatggcttcggctggatcgacatcggcaacgaaaacatctacatcaagtctttcaacaagctgagcctgattatcgaggacaaaagaatcctgagagtgtggcggaagaagtacagcggaaaactcatcaagatcacaaccaagaatagacgggaaatcaccctgacacacgaccatcctgtgtacatcagcaagaccggcgaagtgctggaaatcaacgccgagatggtgaaggtgggagattacatctatatccccaagaacaacaccggctctgccggcagcgccgctggcagcggcatcaacctggacgaggtgatcaaggtcgagacagtggactacaacggccacatctacgacctgaccgttgaggacaaccacacctacatcgccggcaagaacgagggctttgccgtgtccaac

SEQ ID NO: 45 - DNA, 399 bp, unidentified
  source 1..399: mol_type = other DNA
tgtctgagctacgagacagagatcctgaccgtggaatatggcagcctgcctattggcaaaatcgtggaaaagcggatcgagtgcaccgtctacagcgtggacaacaacggaaatatctacacccaacctgtggcccagtggcacgatagaggcgaacaggaggtgttcgagtactgcctggaagatggatctctgatccgggccacaaaggaccacaagttcatgaccgtggacggccagatgctgccaatcgacgagatctttgagcgggaactggacctgatgagagtggataacctgcccaacggcagcgccggctctgccgctggcagcggcgttaaggtgatcggaagacgctccctcggcgtgcagagaatcttcgacatcggcctgagacag

SEQ ID NO: 46 - DNA, 42 bp, unidentified
  source 1..42: mol_type = other DNA
gaccacaacttcctgctggccaacggcgccatcgccgctaat

SEQ ID NO: 47 - DNA, 345 bp, unidentified
  source 1..345: mol_type = other DNA
gggcagagcgcacatcgcccacagtccccgagaagttggggggaggggtcggcaattgaaccggtgcctagagaaggtggcgcggggtaaactgggaaagtgatgtcgtgtactggctccgcctttttcccgagggtgggggagaaccgtatataagtgcagtagtcgccgtgaacgttctttttcgcaacgggtttgccgccagaacacaggtaagtatcaaggttacaagacaggtttaaggagaccaatagaaactgggcttgtcgagacagagaagactcttgcgtttctgataggcacctattggtcttactgacatccactttgcctttctctccacag

SEQ ID NO: 48 - DNA, 392 bp, unidentified
  source 1..392: mol_type = other DNA
gggccccagaagcctggtggttgtttgtccttctcaggggaaaagtgaggcggccccttggaggaaggggccgggcagaatgatctaatcggattccaagcagctcaggggattgtctttttctagcaccttcttgccactcctaagcgtcctccgtgaccccggctgggatttagcctggtgctgtgtcagccccgggctcccaggggcttcccagtggtccccaggaaccctcgacagggccagggcgtctctctcgtccagcaagggcagggacgggccacaggccaagggcgtaagtttagtctttttgtcttttatttcaggtcccggatccggtggtggtgcaaatcaaagaactgctcctcagtggatgttgcctttacttctag

SEQ ID NO: 49 - DNA, 529 bp, unidentified
  source 1..529: mol_type = other DNA
ccattgacgtcaataatgacgtatgttcccatagtaacgccaatagggactttccattgacgtcaatgggtggagtatttacggtaaactgcccacttggcagtacatcaagtgtatcatatgccaagtacgccccctattgacgtcaatgacggtaaatggcccgcctggcattatgcccagtacatgaccttatgggactttcctacttggcagtacatctacgtattagtcatcgctattaccatggtcgaggtgagccccacgttctgcttcactctccccatctcccccccctccccacccccaattttgtatttatttattttttaattattttgtgcagcgatgggggcggggggggggggggggcgcgcgccaggcggggcggggcggggcgaggggcggggcggggcgaggcggagaggtgcggcggcagccaatcagagcggcgcgctccgaaagtttccttttatggcgaggcggcggcggcggcggccctataaaaagcgaagcgcgcggcgggcgg

SEQ ID NO: 50 - DNA, 122 bp, unidentified
  source 1..122: mol_type = other DNA
aacttgtttattgcagcttataatggttacaaataaagcaatagcatcacaaatttcacaaataaagcatttttttcactgcattctagttgtggtttgtccaaactcatcaatgtatctta

SEQ ID NO: 51 - DNA, 225 bp, unidentified
  source 1..225: mol_type = other DNA
ctgtgccttctagttgccagccatctgttgtttgcccctcccccgtgccttccttgaccctggaaggtgccactcccactgtcctttcctaataaaatgaggaaattgcatcgcattgtctgagtaggtgtcattctattctggggggtggggtggggcaggacagcaagggggaggattgggaagacaatagcaggcatgctggggatgcggtgggctctatgg

SEQ ID NO: 52 - DNA, 246 bp, unidentified
  source 1..246: mol_type = other DNA
ataatcaacctctggattacaaaatttgtgaaagattgactggtattcttaactatgttgctccttttacgctatgtggatacgctgctttaatgcctttgtatcatgctattgcttcccgtatggctttcattttctcctccttgtataaatcctggttagttcttgccacggcggaactcatcgccgcctgccttgcccgctgctggacaggggctcggctgttgggcactgacaattccgtgg

SEQ ID NO: 53 - DNA, 250 bp, unidentified
  source 1..250: mol_type = other DNA
ccattgacgtcaataatgacgtatgttcccatagtaacgccaatagggactttccattgacgtcaatgggtggagtatttacggtaaactgcccacttggcagtacatcaagtgtatcatatgccaagtacgccccctattgacgtcaatgacggtaaatggcccgcctggcattatgcccagtacatgaccttatgggactttcctacttggcagtacatctacgtattagtcatcgctattaccatgg

SEQ ID NO: 54 - DNA, 133 bp, Macacine betaherpesvirus 3
  source 1..133: mol_type = other DNA
gtaagtatcaaggttacaagacaggtttaaggagaccaatagaaactgggcttgtcgagacagagaagactcttgcgtttctgataggcacctattggtcttactgacatccactttgcctttctctccacag

SEQ ID NO: 55 - DNA, 97 bp, unidentified
  source 1..97: mol_type = other DNA
gtaagtttagtctttttgtcttttatttcaggtcccggatccggtggtggtgcaaatcaaagaactgctcctcagtggatgttgcctttacttctag

SEQ ID NO: 56 - DNA, 589 bp, unidentified
  source 1..589: mol_type = other DNA
aatcaacctctggattacaaaatttgtgaaagattgactggtattcttaactatgttgctccttttacgctatgtggatacgctgctttaatgcctttgtatcatgctattgcttcccgtatggctttcattttctcctccttgtataaatcctggttgctgtctctttatgaggagttgtggcccgttgtcaggcaacgtggcgtggtgtgcactgtgtttgctgacgcaacccccactggttggggcattgccaccacctgtcagctcctttccgggactttcgctttccccctccctattgccacggcggaactcatcgccgcctgccttgcccgctgctggacaggggctcggctgttgggcactgacaattccgtggtgttgtcggggaaatcatcgtcctttccttggctgctcgcctgtgttgccacctggattctgcgcgggacgtccttctgctacgtcccttcggccctcaatccagcggaccttccttcccgcggcctgctgccggctctgcggcctcttccgcgtcttcgccttcgccctcagacgagtcggatctccctttgggccgcctccccgc

SEQ ID NO: 57 - protein, 199 aa, unidentified
MTEYKPTVRLATRDDVPRAVRTLAAAFADYPATRHTVDPDRHIERVTELQELFLTRVGLDIGKVWVADDGAAVAVWTTPESVEAGAVFAEIGPRMAELSGSRLAAQQQMEGLLAPHRPKEPAWFLATVGVSPDHQGKGLGSAVVLPGVEAAERAGVPAFLETSAPRNLPFYERLGFTVTADVEVPEGPRTWCMTRKPGA

SEQ ID NO: 58 - DNA, 600 bp, unidentified
  source 1..600: mol_type = other DNA
atgaccgagtacaagcccacggtgcgcctcgccacccgcgacgacgtccccagggccgtacgcaccctcgccgccgcgttcgccgactaccccgccacgcgccacaccgtcgatccggaccgccacatcgagcgggtcaccgagctgcaagaactcttcctcacgcgcgtcgggctcgacatcggcaaggtgtgggtcgcggacgacggcgccgcggtggcggtctggaccacgccggagagcgtcgaagcgggggcggtgttcgccgagatcggcccgcgcatggccgagttgagcggttcccggctggccgcgcagcaacagatggaaggcctcctggcgccgcaccggcccaaggagcccgcgtggttcctggccaccgtcggcgtctcgcccgaccaccagggcaagggtctgggcagcgccgtcgtgctccccggagtggaggcggccgagcgcgccggggtgcccgccttcctggagacctccgcgccccgcaacctccccttctacgagcggctcggcttcaccgtcaccgccgacgtcgaggtgcccgaaggaccgcgcacctggtgcatgacccgcaagcccggtgcctga

SEQ ID NO: 59 - DNA, 1175 bp, unidentified
  source 1..1175: mol_type = other DNA
cgtgaggctccggtgcccgtcagtgggcagagcgcacatcgcccacagtccccgagaagttggggggaggggtcggcaattgaaccggtgcctagagaaggtggcgcggggtaaactgggaaagtgatgtcgtgtactggctccgcctttttcccgagggtgggggagaaccgtatataagtgcagtagtcgccgtgaacgttctttttcgcaacgggtttgccgccagaacacaggtaagtgccgtgtgtggttcccgcgggcctggcctctttacgggttatggcccttgcgtgccttgaattacttccacctggctccagtacgtgattcttgatcccgagctggagccaggggcgggccttgcgctttaggagccccttcgcctcgtgcttgagttgaggcctggcctgggcgctggggccgccgcgtgcgaatctggtggcaccttcgcgcctgtctcgctgctttcgataagtctctagccatttaaaatttttgatgacctgctgcgacgctttttttctggcaagatagtcttgtaaatgcgggccaggatctgcacactggtatttcggtttttgggcccgcggccggcgacggggcccgtgcgtcccagcgcacatgttcggcgaggcggggcctgcgagcgcggccaccgagaatcggacgggggtagtctcaagctggccggcctgctctggtgcctggcctcgcgccgccgtgtatcgccccgccctgggcggcaaggctggcccggtcggcaccagttgcgtgagcggaaagatggccgcttcccggccctgctccagggggctcaaaatggaggacgcggcgctcgggagagcgggcgggtgagtcacccacacaaaggaaaagggcctttccgtcctcagccgtcgcttcatgtgactccacggagtaccgggcgccgtccaggcacctcgattagttctggagcttttggagtacgtcgtctttaggttggggggaggggttttatgcgatggagtttccccacactgagtgggtggagactgaagttaggccagcttggcacttgatgtaattctccttggaatttggcctttttgagtttggatcttggttcattctcaagcctcagacagtggttcaaagtttttttcttccatttcaggtgtcgtgaacacgtg

SEQ ID NO: 60 - protein, 154 aa, synthetic construct
CLAGDTLITLADGRRVPIRELVSQQNFSVWALNPQTYRLERARVSRAFCTGIKPVYRLTTRLGRSIRATANHRFLTPQGWKRVDELQPGDYLALPRRIPTASMAAACPELRQLAQSDVYWDPIVSIEPDGVEEVFDLTVPGPHNFVANDIIAHN

SEQ ID NO: 61 - protein, 102 aa, synthetic construct
CLAGDTLITLADGRRVPIRELVSQQNFSVWALNPQTYRLERARVSRAFCTGIKPVYRLTTRLGRSIRATANHRFLTPQGWKRVDELQPGDYLALPRRIPTAS

SEQ ID NO: 62 - protein, 52 aa, synthetic construct
MAAACPELRQLAQSDVYWDPIVSIEPDGVEEVFDLTVPGPHNFVANDIIAHN

SEQ ID NO: 63 - DNA, 306 bp, synthetic construct
  source 1..306: mol_type = other DNA
tgtctggctggcgatactctcattaccctggccgatggacgacgagtgcctattagagaactggtgtcacagcagaatttttccgtgtgggctctgaatcctcagacttaccgcctggagagggctagagtgagtagagctttctgtaccggcatcaaacctgtgtaccgcctcaccactagactggggagatccattagggccactgccaaccaccgatttctcacacctcagggctggaaacgagtcgatgaactccagcctggagattacctggctctgcctaggagaatccctactgcctcc

SEQ ID NO: 64 - DNA, 156 bp, synthetic construct
  source 1..156: mol_type = other DNA
atggcggcggcgtgcccggaactgcgtcagctggcgcagagcgatgtgtattgggatccgattgtgagcattgaaccggatggcgtggaagaagtgtttgatctgaccgtgccgggcccgcataactttgtggcgaacgatattattgcgcataac

SEQ ID NO: 65 - DNA, 48 bp, synthetic construct
  source 1..48: mol_type = other DNA
aataaaggaaatttattttcattgcaatagtgtgttggttttttgtgt

SEQ ID NO: 66 - DNA, 23 bp, synthetic construct
  source 1..23: mol_type = other DNA
aataaaatacgaaatgtgacaga

SEQ ID NO: 67 - DNA, 595 bp, synthetic construct
  source 1..595: mol_type = other DNA
ccattgacgtcaataatgacgtatgttcccatagtaacgccaatagggactttccattgacgtcaatgggtggagtatttacggtaaactgcccacttggcagtacatcaagtgtatcatatgccaagtacgccccctattgacgtcaatgacggtaaatggcccgcctggcattatgcccagtacatgaccttatgggactttcctacttggcagtacatctacgtattagtcatcgctattaccatgggggcagagcgcacatcgcccacagtccccgagaagttggggggaggggtcggcaattgaaccggtgcctagagaaggtggcgcggggtaaactgggaaagtgatgtcgtgtactggctccgcctttttcccgagggtgggggagaaccgtatataagtgcagtagtcgccgtgaacgttctttttcgcaacgggtttgccgccagaacacaggtaagtatcaaggttacaagacaggtttaaggagaccaatagaaactgggcttgtcgagacagagaagactcttgcgtttctgataggcacctattggtcttactgacatccactttgcctttctctccacag

SEQ ID NO: 68 - DNA, 642 bp, synthetic construct
  source 1..642: mol_type = other DNA
ccattgacgtcaataatgacgtatgttcccatagtaacgccaatagggactttccattgacgtcaatgggtggagtatttacggtaaactgcccacttggcagtacatcaagtgtatcatatgccaagtacgccccctattgacgtcaatgacggtaaatggcccgcctggcattatgcccagtacatgaccttatgggactttcctacttggcagtacatctacgtattagtcatcgctattaccatgggggccccagaagcctggtggttgtttgtccttctcaggggaaaagtgaggcggccccttggaggaaggggccgggcagaatgatctaatcggattccaagcagctcaggggattgtctttttctagcaccttcttgccactcctaagcgtcctccgtgaccccggctgggatttagcctggtgctgtgtcagccccgggctcccaggggcttcccagtggtccccaggaaccctcgacagggccagggcgtctctctcgtccagcaagggcagggacgggccacaggccaagggcgtaagtttagtctttttgtcttttatttcaggtcccggatccggtggtggtgcaaatcaaagaactgctcctcagtggatgttgcctttacttctag

SEQ ID NO: 69 - DNA, 428 bp, synthetic construct
  source 1..428: mol_type = other DNA
gggccccagaagcctggtggttgtttgtccttctcaggggaaaagtgaggcggccccttggaggaaggggccgggcagaatgatctaatcggattccaagcagctcaggggattgtctttttctagcaccttcttgccactcctaagcgtcctccgtgaccccggctgggatttagcctggtgctgtgtcagccccgggctcccaggggcttcccagtggtccccaggaaccctcgacagggccagggcgtctctctcgtccagcaagggcagggacgggccacaggccaagggcgtaagtatcaaggttacaagacaggtttaaggagaccaatagaaactgggcttgtcgagacagagaagactcttgcgtttctgataggcacctattggtcttactgacatccactttgcctttctctccacag

SEQ ID NO: 70 - DNA, 678 bp, synthetic construct
  source 1..678: mol_type = other DNA
ccattgacgtcaataatgacgtatgttcccatagtaacgccaatagggactttccattgacgtcaatgggtggagtatttacggtaaactgcccacttggcagtacatcaagtgtatcatatgccaagtacgccccctattgacgtcaatgacggtaaatggcccgcctggcattatgcccagtacatgaccttatgggactttcctacttggcagtacatctacgtattagtcatcgctattaccatgggggccccagaagcctggtggttgtttgtccttctcaggggaaaagtgaggcggccccttggaggaaggggccgggcagaatgatctaatcggattccaagcagctcaggggattgtctttttctagcaccttcttgccactcctaagcgtcctccgtgaccccggctgggatttagcctggtgctgtgtcagccccgggctcccaggggcttcccagtggtccccaggaaccctcgacagggccagggcgtctctctcgtccagcaagggcagggacgggccacaggccaagggcgtaagtatcaaggttacaagacaggtttaaggagaccaatagaaactgggcttgtcgagacagagaagactcttgcgtttctgataggcacctattggtcttactgacatccactttgcctttctctccacag